European Patent Specification EP 3 177 307 B1, published July 17, 2024. Title: INTERLEUKIN-2/INTERLEUKIN-2 RECEPTOR ALPHA FUSION PROTEINS AND METHODS OF USE. Applicant: Malek, Thomas. The sequence listing filed with the application follows.

SEQUENCE LISTING (65 sequences)

SEQ ID NO: 1 - protein, 153 aa, Homo sapeins
MYRMQLLSCIALSLALVTNSAPTSSSTKKTQLQLEHLLLDLQMILNGINNYKNPKLTRMLTFKFYMPKKATELKHLQCLEEELKPLEEVLNLAQSKNFHLRPRDLISNINVIVLELKGSETTFMCEYADETATIVEFLNRWITFCQSIISTLT

SEQ ID NO: 2 - protein, 133 aa, Homo sapiens [sequence omitted]

SEQ ID NO: 3 - protein, 169 aa, Mus musculus
MYSMQLASCVTLTLVLLVNSAPTSSSTSSSTAEAQQQQQQQQQQQQHLEQLLMDLQELLSRMENYRNLKLPRMLTFKFYLPKQATELKDLQCLEDELGPLRHVLDLTQSKSFQLEDAENFISNIRVTVVKLKGSDNTFECQFDDESATVVDFLRRWIAFCQSIISTSPQ

SEQ ID NO: 4 - protein, 149 aa, Mus musculus
APTSSSTSSSTAEAQQQQQQQQQQQQHLEQLLMDLQELLSRMENYRNLKLPRMLTFKFYLPKQATELKDLQCLEDELGPLRHVLDLTQSKSFQLEDAENFISNIRVTVVKLKGSDNTFECQFDDESATVVDFLRRWIAFCQSIISTSPQ

SEQ ID NO: 5 - protein, 272 aa, Homo sapiens
MDSYLLMWGLLTFIMVPGCQAELCDDDPPEIPHATFKAMAYKEGTMLNCECKRGFRRIKSGSLYMLCTGNSSHSSWDNQCQCTSSATRNTTKQVTPQPEEQKERKTTEMQSPMQPVDQASLPGHCREPPPWENEATERIYHFVVGQMVYYQCVQGYRALHRGPAESVCKMTHGKTRWTQPQLICTGEMETSQFPGEEKPQASPEGRPESETSCLVTTTDFQIQTEMAATMETSIFTTEYQVAVAGCVFLLISVLLLSGLTWQRRQRKSRRTI

SEQ ID NO: 6 - protein, 251 aa, Homo sapiens
ELCDDDPPEIPHATFKAMAYKEGTMLNCECKRGFRRIKSGSLYMLCTGNSSHSSWDNQCQCTSSATRNTTKQVTPQPEEQKERKTTEMQSPMQPVDQASLPGHCREPPPWENEATERIYHFVVGQMVYYQCVQGYRALHRGPAESVCKMTHGKTRWTQPQLICTGEMETSQFPGEEKPQASPEGRPESETSCLVTTTDFQIQTEMAATMETSIFTTEYQVAVAGCVFLLISVLLLSGLTWQRRQRKSRRTI

SEQ ID NO: 7 - protein, 219 aa, Homo sapiens
ELCDDDPPEIPHATFKAMAYKEGTMLNCECKRGFRRIKSGSLYMLCTGNSSHSSWDNQCQCTSSATRNTTKQVTPQPEEQKERKTTEMQSPMQPVDQASLPGHCREPPPWENEATERIYHFVVGQMVYYQCVQGYRALHRGPAESVCKMTHGKTRWTQPQLICTGEMETSQFPGEEKPQASPEGRPESETSCLVTTTDFQIQTEMAATMETSIFTTEYQ

SEQ ID NO: 8 - protein, 268 aa, Mus musculus
MEPRLLMLGFLSLTIVPSCRAELCLYDPPEVPNATFKALSYKNGTILNCECKRGFRRLKELVYMRCLGNSWSSNCQCTSNSHDKSRKQVTAQLEHQKEQQTTTDMQKPTQSMHQENLTGHCREPPPWKHEDSKRIYHFVEGQSVHYECIPGYKALQRGPAISICKMKCGKTGWTQPQLTCVDEREHHRFLASEESQGSRNSSPESETSCPITTTDFPQPTETTAMTETFVLTMEYKVAVASCLFLLISILLLSGLTWQHRWRKSRRTI

SEQ ID NO: 9 - protein, 247 aa, Mus musculus
ELCLYDPPEVPNATFKALSYKNGTILNCECKRGFRRLKELVYMRCLGNSWSSNCQCTSNSHDKSRKQVTAQLEHQKEQQTTTDMQKPTQSMHQENLTGHCREPPPWKHEDSKRIYHFVEGQSVHYECIPGYKALQRGPAISICKMKCGKTGWTQPQLTCVDEREHHRFLASEESQGSRNSSPESETSCPITTTDFPQPTETTAMTETFVLTMEYKVAVASCLFLLISILLLSGLTWQHRWRKSRRTI

SEQ ID NO: 10 - protein, 215 aa, Mus musculus
ELCLYDPPEVPNATFKALSYKNGTILNCECKRGFRRLKELVYMRCLGNSWSSNCQCTSNSHDKSRKQVTAQLEHQKEQQTTTDMQKPTQSMHQENLTGHCREPPPWKHEDSKRIYHFVEGQSVHYECIPGYKALQRGPAISICKMKCGKTGWTQPQLTCVDEREHHRFLASEESQGSRNSSPESETSCPITTTDFPQPTETTAMTETFVLTMEYK

SEQ ID NO: 11 - protein, 16 aa, Artificial Sequence
  (Gly3Ser)4 linker
GGGSGGGSGGGSGGGS

SEQ ID NO: 12 - protein, 8 aa, Artificial Sequence
  (Gly3Ser)2 linker
GGGSGGGS

SEQ ID NO: 13 - protein, 12 aa, Artificial Sequence
  (Gly3Ser)3 linker
GGGSGGGSGGGS

SEQ ID NO: 14 - protein, 20 aa, Artificial Sequence
  (Gly3Ser)5 linker
GGGSGGGSGGGSGGGSGGGS

SEQ ID NO: 15 - protein, 3 aa, Artificial Sequence
  Gly3 linker
GGG

SEQ ID NO: 16 - protein, 384 aa, Artificial Sequence
  Synthesized Mature form of IL-2 (Gly4Ser)4-extracellular domain of IL-2 R
APTSSSTSSSTAEAQQQQQQQQQQQQHLEQLLMDLQELLSRMENYRNLKLPRMLTFKFYLPKQATELKDLQCLEDELGPLRHVLDLTQSKSFQLEDAENFISNIRVTVVKLKGSDNTFECQFDDESATVVDFLRRWIAFCQSIISTSPQGGGGSGGGGSGGGGSGGGGSELCLYDPPEVPNATFKALSYKNGTILNCECKRGFRRLKELVYMRCLGNSWSSNCQCTSNSHDKSRKQVTAQLEHQKEQQTTTDMQKPTQSMHQENLTGHCREPPPWKHEDSKRIYHFVEGQSVHYECIPGYKALQRGPAISICKMKCGKTGWTQPQLTCVDEREHHRFLASEESQGSRNSSPESETSCPITTTDFPQPTETTAMTETFVLTMEYK

SEQ ID NO: 17 - protein, 404 aa, Artificial Sequence
  Synthesized unprocessed form of IL-2 (Gly4Ser)4-extracellular domain of IL-2 R
MDSMQLASCVTLTLVLLVNSAPTSSSTSSSTAEAQQQQQQQQQQQQHLEQLLMDLQELLSRMENYRNLKLPRMLTFKFYLPKQATELKDLQCLEDELGPLRHVLDLTQSKSFQLEDAENFISNIRVTVVKLKGSDNTFECQFDDESATVVDFLRRWIAFCQSIISTSPQGGGGSGGGGSGGGGSGGGGSELCLYDPPEVPNATFKALSYKNGTILNCECKRGFRRLKELVYMRCLGNSWSSNCQCTSNSHDKSRKQVTAQLEHQKEQQTTTDMQKPTQSMHQENLTGHCREPPPWKHEDSKRIYHFVEGQSVHYECIPGYKALQRGPAISICKMKCGKTGWTQPQLTCVDEREHHRFLASEESQGSRNSSPESETSCPITTTDFPQPTETTAMTETFVLTMEYK

SEQ ID NO: 18 - protein, 389 aa, Artificial Sequence
  Synthesized mature form of IL-2 (Gly4Ser)5- extracellular domain of IL-2 R
APTSSSTSSSTAEAQQQQQQQQQQQQHLEQLLMDLQELLSRMENYRNLKLPRMLTFKFYLPKQATELKDLQCLEDELGPLRHVLDLTQSKSFQLEDAENFISNIRVTVVKLKGSDNTFECQFDDESATVVDFLRRWIAFCQSIISTSPQGGGGSGGGGSGGGGSGGGGSGGGGSELCLYDPPEVPNATFKALSYKNGTILNCECKRGFRRLKELVYMRCLGNSWSSNCQCTSNSHDKSRKQVTAQLEHQKEQQTTTDMQKPTQSMHQENLTGHCREPPPWKHEDSKRIYHFVEGQSVHYECIPGYKALQRGPAISICKMKCGKTGWTQPQLTCVDEREHHRFLASEESQGSRNSSPESETSCPITTTDFPQPTETTAMTETFVLTMEYK

SEQ ID NO: 19 - protein, 409 aa, Artificial Sequence
  Synthesized unprocessed form of IL-2 (Gly4Ser)5- extracellular domain of IL-2 R
MDSMQLASCVTLTLVLLVNSAPTSSSTSSSTAEAQQQQQQQQQQQQHLEQLLMDLQELLSRMENYRNLKLPRMLTFKFYLPKQATELKDLQCLEDELGPLRHVLDLTQSKSFQLEDAENFISNIRVTVVKLKGSDNTFECQFDDESATVVDFLRRWIAFCQSIISTSPQGGGGSGGGGSGGGGSGGGGSGGGGSELCLYDPPEVPNATFKALSYKNGTILNCECKRGFRRLKELVYMRCLGNSWSSNCQCTSNSHDKSRKQVTAQLEHQKEQQTTTDMQKPTQSMHQENLTGHCREPPPWKHEDSKRIYHFVEGQSVHYECIPGYKALQRGPAISICKMKCGKTGWTQPQLTCVDEREHHRFLASEESQGSRNSSPESETSCPITTTDFPQPTETTAMTETFVLTMEYK

SEQ ID NO: 20 - protein, 380 aa, Artificial Sequence
  Synthesized mature form of IL-2 (Gly3Ser)4- extracellular domain of IL-2 R
APTSSSTSSSTAEAQQQQQQQQQQQQHLEQLLMDLQELLSRMENYRNLKLPRMLTFKFYLPKQATELKDLQCLEDELGPLRHVLDLTQSKSFQLEDAENFISNIRVTVVKLKGSDNTFECQFDDESATVVDFLRRWIAFCQSIISTSPQGGGSGGGSGGGSGGGSELCLYDPPEVPNATFKALSYKNGTILNCECKRGFRRLKELVYMRCLGNSWSSNCQCTSNSHDKSRKQVTAQLEHQKEQQTTTDMQKPTQSMHQENLTGHCREPPPWKHEDSKRIYHFVEGQSVHYECIPGYKALQRGPAISICKMKCGKTGWTQPQLTCVDEREHHRFLASEESQGSRNSSPESETSCPITTTDFPQPTETTAMTETFVLTMEYK

SEQ ID NO: 21 - protein, 400 aa, Artificial Sequence
  Synthesized unprocessed form of IL-2 (Gly3Ser)4- extracellular domain of IL-2 R
MDSMQLASCVTLTLVLLVNSAPTSSSTSSSTAEAQQQQQQQQQQQQHLEQLLMDLQELLSRMENYRNLKLPRMLTFKFYLPKQATELKDLQCLEDELGPLRHVLDLTQSKSFQLEDAENFISNIRVTVVKLKGSDNTFECQFDDESATVVDFLRRWIAFCQSIISTSPQGGGSGGGSGGGSGGGSELCLYDPPEVPNATFKALSYKNGTILNCECKRGFRRLKELVYMRCLGNSWSSNCQCTSNSHDKSRKQVTAQLEHQKEQQTTTDMQKPTQSMHQENLTGHCREPPPWKHEDSKRIYHFVEGQSVHYECIPGYKALQRGPAISICKMKCGKTGWTQPQLTCVDEREHHRFLASEESQGSRNSSPESETSCPITTTDFPQPTETTAMTETFVLTMEYK

SEQ ID NO: 22 - protein, 372 aa, Artificial Sequence
  Synthesized mature form IL-2 (Gly4Ser)4- extracellular domain of IL-2 R
APTSSSTKKTQLQLEHLLLDLQMILNGINNYKNPKLTRMLTFKFYMPKKATELKHLQCLEEELKPLEEVLNLAQSKNFHLRPRDLISNINVIVLELKGSETTFMCEYADETATIVEFLNRWITFCQSIISTLTGGGGSGGGGSGGGGSGGGGSELCDDDPPEIPHATFKAMAYKEGTMLNCECKRGFRRIKSGSLYMLCTGNSSHSSWDNQCQCTSSATRNTTKQVTPQPEEQKERKTTEMQSPMQPVDQASLPGHCREPPPWENEATERIYHFVVGQMVYYQCVQGYRALHRGPAESVCKMTHGKTRWTQPQLICTGEMETSQFPGEEKPQASPEGRPESETSCLVTTTDFQIQTEMAATMETSIFTTEYQ

SEQ ID NO: 23 - protein, 392 aa, Artificial Sequence
  Synthesized unprocessed form IL-2 (Gly4Ser)4- extracellular domain of IL-2 R
MDRMQLLSCIALSLALVTNSAPTSSSTKKTQLQLEHLLLDLQMILNGINNYKNPKLTRMLTFKFYMPKKATELKHLQCLEEELKPLEEVLNLAQSKNFHLRPRDLISNINVIVLELKGSETTFMCEYADETATIVEFLNRWITFCQSIISTLTGGGGSGGGGSGGGGSGGGGSELCDDDPPEIPHATFKAMAYKEGTMLNCECKRGFRRIKSGSLYMLCTGNSSHSSWDNQCQCTSSATRNTTKQVTPQPEEQKERKTTEMQSPMQPVDQASLPGHCREPPPWENEATERIYHFVVGQMVYYQCVQGYRALHRGPAESVCKMTHGKTRWTQPQLICTGEMETSQFPGEEKPQASPEGRPESETSCLVTTTDFQIQTEMAATMETSIFTTEYQ

SEQ ID NO: 24 - protein, 368 aa, Artificial Sequence
  Synthesized mature form IL-2 (Gly3Ser)4- extracellular domain of IL-2 R
APTSSSTKKTQLQLEHLLLDLQMILNGINNYKNPKLTRMLTFKFYMPKKATELKHLQCLEEELKPLEEVLNLAQSKNFHLRPRDLISNINVIVLELKGSETTFMCEYADETATIVEFLNRWITFCQSIISTLTGGGSGGGSGGGSGGGSELCDDDPPEIPHATFKAMAYKEGTMLNCECKRGFRRIKSGSLYMLCTGNSSHSSWDNQCQCTSSATRNTTKQVTPQPEEQKERKTTEMQSPMQPVDQASLPGHCREPPPWENEATERIYHFVVGQMVYYQCVQGYRALHRGPAESVCKMTHGKTRWTQPQLICTGEMETSQFPGEEKPQASPEGRPESETSCLVTTTDFQIQTEMAATMETSIFTTEYQ

SEQ ID NO: 25 - protein, 388 aa, Artificial Sequence
  Synthesized unprocessed form IL-2 (Gly3Ser)4- extracellular domain of IL-2 R
MDRMQLLSCIALSLALVTNSAPTSSSTKKTQLQLEHLLLDLQMILNGINNYKNPKLTRMLTFKFYMPKKATELKHLQCLEEELKPLEEVLNLAQSKNFHLRPRDLISNINVIVLELKGSETTFMCEYADETATIVEFLNRWITFCQSIISTLTGGGSGGGSGGGSGGGSELCDDDPPEIPHATFKAMAYKEGTMLNCECKRGFRRIKSGSLYMLCTGNSSHSSWDNQCQCTSSATRNTTKQVTPQPEEQKERKTTEMQSPMQPVDQASLPGHCREPPPWENEATERIYHFVVGQMVYYQCVQGYRALHRGPAESVCKMTHGKTRWTQPQLICTGEMETSQFPGEEKPQASPEGRPESETSCLVTTTDFQIQTEMAATMETSIFTTEYQ

SEQ ID NO: 26 - protein, 364 aa, Artificial Sequence
  Synthesized mature form IL-2 (Gly3Ser)3- extracellular domain of IL-2 R
APTSSSTKKTQLQLEHLLLDLQMILNGINNYKNPKLTRMLTFKFYMPKKATELKHLQCLEEELKPLEEVLNLAQSKNFHLRPRDLISNINVIVLELKGSETTFMCEYADETATIVEFLNRWITFCQSIISTLTGGGSGGGSGGGSELCDDDPPEIPHATFKAMAYKEGTMLNCECKRGFRRIKSGSLYMLCTGNSSHSSWDNQCQCTSSATRNTTKQVTPQPEEQKERKTTEMQSPMQPVDQASLPGHCREPPPWENEATERIYHFVVGQMVYYQCVQGYRALHRGPAESVCKMTHGKTRWTQPQLICTGEMETSQFPGEEKPQASPEGRPESETSCLVTTTDFQIQTEMAATMETSIFTTEYQ

SEQ ID NO: 27 - protein, 384 aa, Artificial Sequence
  Synthesized unprocessed form of IL-2 (Gly3Ser)3- extracellular domain of IL-2 R
MDRMQLLSCIALSLALVTNSAPTSSSTKKTQLQLEHLLLDLQMILNGINNYKNPKLTRMLTFKFYMPKKATELKHLQCLEEELKPLEEVLNLAQSKNFHLRPRDLISNINVIVLELKGSETTFMCEYADETATIVEFLNRWITFCQSIISTLTGGGSGGGSGGGSELCDDDPPEIPHATFKAMAYKEGTMLNCECKRGFRRIKSGSLYMLCTGNSSHSSWDNQCQCTSSATRNTTKQVTPQPEEQKERKTTEMQSPMQPVDQASLPGHCREPPPWENEATERIYHFVVGQMVYYQCVQGYRALHRGPAESVCKMTHGKTRWTQPQLICTGEMETSQFPGEEKPQASPEGRPESETSCLVTTTDFQIQTEMAATMETSIFTTEYQ

SEQ ID NO: 28 - DNA, 66 bp, Artificial Sequence
  IL-2 leader optimized Kozak sequence
gccaccatggacaggatgcaactcctgtcttgcattgcactaagtcttgcacttgtcacaaacagt

SEQ ID NO: 29 - DNA, 1239 bp, Artificial Sequence
  Synthesized unprocessed form of IL-2 (Gly4Ser)4-extracellular domain of IL-2 R
atggacagcatgcagctcgcatcctgtgtcacattgacacttgtgctccttgtcaacagcgcacccacttcaagctctacttcaagctctacagcggaagcacagcagcagcagcagcagcagcagcagcagcagcacctggagcagctgttgatggacctacaggagctcctgagcaggatggagaattacaggaacctgaaactccccaggatgctcaccttcaaattttacttgcccaagcaggccacagaattgaaagatcttcagtgcctagaagatgaacttggacctctgcggcatgttctggatttgactcaaagcaaaagctttcaattggaagatgctgagaatttcatcagcaatatcagagtaactgttgtaaaactaaagggctctgacaacacatttgagtgccaattcgatgatgagtcagcaactgtggtggactttctgaggagatggatagccttctgtcaaagcatcatctcaacaagccctcaaggtggaggtggatctggtggaggtggatcaggtggaggtggatccggtggaggtggatctgaactgtgtctgtatgacccacccgaggtccccaatgccacattcaaagccctctcctacaagaacggcaccatcctaaactgtgaatgcaagagaggtttccgaagactaaaggaattggtctatatgcgttgcttaggaaactcctggagcagcaactgccagtgcaccagcaactcccatgacaaatcgagaaagcaagttacagctcaacttgaacaccagaaagagcaacaaaccacaacagacatgcagaagccaacacagtctatgcaccaagagaaccttacaggtcactgcagggagccacctccttggaaacatgaagattccaagagaatctatcatttcgtggaaggacagagtgttcactacgagtgtattccgggatacaaggctctacagagaggtcctgctattagcatctgcaagatgaagtgtgggaaaacggggtggactcagccccagctcacatgtgtagatgaaagagaacaccaccgatttctggctagtgaggaatctcaaggaagcagaaattcttctcccgagagtgagacttcctgccccataaccaccacagacttcccacaacccacagaaacaactgcaatgacggagacatttgtgctcacaatggagtataagggtggacatcaccatcaccatcactaataa

SEQ ID NO: 30 - DNA, 1227 bp, Artificial Sequence
  Synthesized unprocessed form of IL-2 (Gly3Ser)4- extracellular domain of IL-2 R
atggacagcatgcagctcgcatcctgtgtcacattgacacttgtgctccttgtcaacagcgcacccacttcaagctctacttcaagctctacagcggaagcacagcagcagcagcagcagcagcagcagcagcagcacctggagcagctgttgatggacctacaggagctcctgagcaggatggagaattacaggaacctgaaactccccaggatgctcaccttcaaattttacttgcccaagcaggccacagaattgaaagatcttcagtgcctagaagatgaacttggacctctgcggcatgttctggatttgactcaaagcaaaagctttcaattggaagatgctgagaatttcatcagcaatatcagagtaactgttgtaaaactaaagggctctgacaacacatttgagtgccaattcgatgatgagtcagcaactgtggtggactttctgaggagatggatagccttctgtcaaagcatcatctcaacaagccctcaaggtggaggttctggtggaggttcaggtggaggttcgggtggaggttctgaactgtgtctgtatgacccacccgaggtccccaatgccacattcaaagccctctcctacaagaacggcaccatcctaaactgtgaatgcaagagaggtttccgaagactaaaggaattggtctatatgcgttgcttaggaaactcctggagcagcaactgccagtgcaccagcaactcccatgacaaatcgagaaagcaagttacagctcaacttgaacaccagaaagagcaacaaaccacaacagacatgcagaagccaacacagtctatgcaccaagagaaccttacaggtcactgcagggagccacctccttggaaacatgaagattccaagagaatctatcatttcgtggaaggacagagtgttcactacgagtgtattccgggatacaaggctctacagagaggtcctgctattagcatctgcaagatgaagtgtgggaaaacggggtggactcagccccagctcacatgtgtagatgaaagagaacaccaccgatttctggctagtgaggaatctcaaggaagcagaaattcttctcccgagagtgagacttcctgccccataaccaccacagacttcccacaacccacagaaacaactgcaatgacggagacatttgtgctcacaatggagtataagggtggacatcaccatcaccatcactaataa

SEQ ID NO: 31 - DNA, 1254 bp, Artificial Sequence
  Synthesized unprocessed form of IL-2 (Gly4Ser)5- extracellular domain of IL-2 R
atggacagcatgcagctcgcatcctgtgtcacattgacacttgtgctccttgtcaacagcgcacccacttcaagctctacttcaagctctacagcggaagcacagcagcagcagcagcagcagcagcagcagcagcacctggagcagctgttgatggacctacaggagctcctgagcaggatggagaattacaggaacctgaaactccccaggatgctcaccttcaaattttacttgcccaagcaggccacagaattgaaagatcttcagtgcctagaagatgaacttggacctctgcggcatgttctggatttgactcaaagcaaaagctttcaattggaagatgctgagaatttcatcagcaatatcagagtaactgttgtaaaactaaagggctctgacaacacatttgagtgccaattcgatgatgagtcagcaactgtggtggactttctgaggagatggatagccttctgtcaaagcatcatctcaacaagccctcaaggtggaggtggatcaggtggaggtggatctggtggaggtggatcaggtggaggtggatccggtggaggtggatctgaactgtgtctgtatgacccacccgaggtccccaatgccacattcaaagccctctcctacaagaacggcaccatcctaaactgtgaatgcaagagaggtttccgaagactaaaggaattggtctatatgcgttgcttaggaaactcctggagcagcaactgccagtgcaccagcaactcccatgacaaatcgagaaagcaagttacagctcaacttgaacaccagaaagagcaacaaaccacaacagacatgcagaagccaacacagtctatgcaccaagagaaccttacaggtcactgcagggagccacctccttggaaacatgaagattccaagagaatctatcatttcgtggaaggacagagtgttcactacgagtgtattccgggatacaaggctctacagagaggtcctgctattagcatctgcaagatgaagtgtgggaaaacggggtggactcagccccagctcacatgtgtagatgaaagagaacaccaccgatttctggctagtgaggaatctcaaggaagcagaaattcttctcccgagagtgagacttcctgccccataaccaccacagacttcccacaacccacagaaacaactgcaatgacggagacatttgtgctcacaatggagtataagggtggacatcaccatcaccatcactaataa

SEQ ID NO: 32 - DNA, 1206 bp, Artificial Sequence
  Synthesized unprocessed form IL-2 (Gly4Ser)4- extracellular domain of IL-2 R
atggacaggatgcaactcctgtcttgcattgcactaagtcttgcacttgtcacaaacagtgcacctacttcaagttctacaaagaaaacacagctacaactggagcatttactgctggatttacagatgattttgaatggaattaataattacaagaatcccaaactcaccaggatgctcacatttaagttttacatgcccaagaaggccacagaactgaaacatcttcagtgtctagaagaagaactcaaacctctggaggaagtgctaaatttagctcaaagcaaaaactttcacttaagacccagggacttaatcagcaatatcaacgtaatagttctggaactaaagggatctgaaacaacattcatgtgtgaatatgctgatgagacagcaaccattgtagaatttctgaacagatggattaccttttgtcaaagcatcatctcaacactgactggtggaggtggatctggtggaggtggatcaggtggaggtggatccggtggaggtggatctgagctctgtgacgatgacccgccagagatcccacacgccacattcaaagccatggcctacaaggaaggaaccatgttgaactgtgaatgcaagagaggtttccgcagaataaaaagcgggtcactctatatgctctgtacaggaaactctagccactcgtcctgggacaaccaatgtcaatgcacaagctctgccactcggaacacaacgaaacaagtgacacctcaacctgaagaacagaaagaaaggaaaaccacagaaatgcaaagtccaatgcagccagtggaccaagcgagccttccaggtcactgcagggaacctccaccatgggaaaatgaagccacagagagaatttatcatttcgtggtggggcagatggtttattatcagtgcgtccagggatacagggctctacacagaggtcctgctgagagcgtctgcaaaatgacccacgggaagacaaggtggacccagccccagctcatatgcacaggtgaaatggagaccagtcagtttccaggtgaagagaagcctcaggcaagccccgaaggccgtcctgagagtgagacttcctgcctcgtcacaacaacagattttcaaatacagacagaaatggctgcaaccatggagacgtccatatttacaacagagtaccagggtggacatcaccatcaccatcactaataa

SEQ ID NO: 33 - DNA, 1194 bp, Artificial Sequence
  Synthesized unprocessed form IL-2 (Gly3Ser)4- extracellular domain of IL-2 R
atggacaggatgcaactcctgtcttgcattgcactaagtcttgcacttgtcacaaacagtgcacctacttcaagttctacaaagaaaacacagctacaactggagcatttactgctggatttacagatgattttgaatggaattaataattacaagaatcccaaactcaccaggatgctcacatttaagttttacatgcccaagaaggccacagaactgaaacatcttcagtgtctagaagaagaactcaaacctctggaggaagtgctaaatttagctcaaagcaaaaactttcacttaagacccagggacttaatcagcaatatcaacgtaatagttctggaactaaagggatctgaaacaacattcatgtgtgaatatgctgatgagacagcaaccattgtagaatttctgaacagatggattaccttttgtcaaagcatcatctcaacactgactggtggaggttctggtggaggttcaggtggaggttcgggtggaggttctgagctctgtgacgatgacccgccagagatcccacacgccacattcaaagccatggcctacaaggaaggaaccatgttgaactgtgaatgcaagagaggtttccgcagaataaaaagcgggtcactctatatgctctgtacaggaaactctagccactcgtcctgggacaaccaatgtcaatgcacaagctctgccactcggaacacaacgaaacaagtgacacctcaacctgaagaacagaaagaaaggaaaaccacagaaatgcaaagtccaatgcagccagtggaccaagcgagccttccaggtcactgcagggaacctccaccatgggaaaatgaagccacagagagaatttatcatttcgtggtggggcagatggtttattatcagtgcgtccagggatacagggctctacacagaggtcctgctgagagcgtctgcaaaatgacccacgggaagacaaggtggacccagccccagctcatatgcacaggtgaaatggagaccagtcagtttccaggtgaagagaagcctcaggcaagccccgaaggccgtcctgagagtgagacttcctgcctcgtcacaacaacagattttcaaatacagacagaaatggctgcaaccatggagacgtccatatttacaacagagtaccagggtggacatcaccatcaccatcactaataa

SEQ ID NO: 34 - DNA, 1182 bp, Artificial Sequence
  Synthesized unprocessed form of IL-2 (Gly3Ser)3- extracellular domain of IL-2 R
atggacaggatgcaactcctgtcttgcattgcactaagtcttgcacttgtcacaaacagtgcacctacttcaagttctacaaagaaaacacagctacaactggagcatttactgctggatttacagatgattttgaatggaattaataattacaagaatcccaaactcaccaggatgctcacatttaagttttacatgcccaagaaggccacagaactgaaacatcttcagtgtctagaagaagaactcaaacctctggaggaagtgctaaatttagctcaaagcaaaaactttcacttaagacccagggacttaatcagcaatatcaacgtaatagttctggaactaaagggatctgaaacaacattcatgtgtgaatatgctgatgagacagcaaccattgtagaatttctgaacagatggattaccttttgtcaaagcatcatctcaacactgactggtggaggttctggtggaggttcaggtggaggttcggagctctgtgacgatgacccgccagagatcccacacgccacattcaaagccatggcctacaaggaaggaaccatgttgaactgtgaatgcaagagaggtttccgcagaataaaaagcgggtcactctatatgctctgtacaggaaactctagccactcgtcctgggacaaccaatgtcaatgcacaagctctgccactcggaacacaacgaaacaagtgacacctcaacctgaagaacagaaagaaaggaaaaccacagaaatgcaaagtccaatgcagccagtggaccaagcgagccttccaggtcactgcagggaacctccaccatgggaaaatgaagccacagagagaatttatcatttcgtggtggggcagatggtttattatcagtgcgtccagggatacagggctctacacagaggtcctgctgagagcgtctgcaaaatgacccacgggaagacaaggtggacccagccccagctcatatgcacaggtgaaatggagaccagtcagtttccaggtgaagagaagcctcaggcaagccccgaaggccgtcctgagagtgagacttcctgcctcgtcacaacaacagattttcaaatacagacagaaatggctgcaaccatggagacgtccatatttacaacagagtaccagggtggacatcaccatcaccatcactaataa

SEQ ID NO: 35 - DNA, 13 bp, Artificial Sequence
  Kozak consensus
gccgccrccaugg

SEQ ID NO: 36 - protein, 396 aa, Artificial Sequence
  Synthesized unprocessed form of IL-2 (Gly3Ser)3- extracellular domain of IL-2 R
MYSMQLASCVTLTLVLLVNSAPTSSSTSSSTAEAQQQQQQQQQQQQHLEQLLMDLQELLSRMENYRNLKLPRMLTFKFYLPKQATELKDLQCLEDELGPLRHVLDLTQSKSFQLEDAENFISNIRVTVVKLKGSDNTFECQFDDESATVVDFLRRWIAFCQSIISTSPQGGGSGGGSGGGSELCLYDPPEVPNATFKALSYKNGTILNCECKRGFRRLKELVYMRCLGNSWSSNCQCTSNSHDKSRKQVTAQLEHQKEQQTTTDMQKPTQSMHQENLTGHCREPPPWKHEDSKRIYHFVEGQSVHYECIPGYKALQRGPAISICKMKCGKTGWTQPQLTCVDEREHHRFLASEESQGSRNSSPESETSCPITTTDFPQPTETTAMTETFVLTMEYK

SEQ ID NO: 37 - protein, 396 aa, Artificial Sequence
  Synthesized mature form of IL-2 (Gly3Ser)3- extracellular domain of IL-2 R
MDSMQLASCVTLTLVLLVNSAPTSSSTSSSTAEAQQQQQQQQQQQQHLEQLLMDLQELLSRMENYRNLKLPRMLTFKFYLPKQATELKDLQCLEDELGPLRHVLDLTQSKSFQLEDAENFISNIRVTVVKLKGSDNTFECQFDDESATVVDFLRRWIAFCQSIISTSPQGGGSGGGSGGGSELCLYDPPEVPNATFKALSYKNGTILNCECKRGFRRLKELVYMRCLGNSWSSNCQCTSNSHDKSRKQVTAQLEHQKEQQTTTDMQKPTQSMHQENLTGHCREPPPWKHEDSKRIYHFVEGQSVHYECIPGYKALQRGPAISICKMKCGKTGWTQPQLTCVDEREHHRFLASEESQGSRNSSPESETSCPITTTDFPQPTETTAMTETFVLTMEYK

SEQ ID NO: 38 - protein, 397 aa, Artificial Sequence
  Synthesized unprocessed form of IL-2 (Gly4Ser)5- extracellular domain of IL-2 R
MDRMQLLSCIALSLALVTNSAPTSSSTKKTQLQLEHLLLDLQMILNGINNYKNPKLTRMLTFKFYMPKKATELKHLQCLEEELKPLEEVLNLAQSKNFHLRPRDLISNINVIVLELKGSETTFMCEYADETATIVEFLNRWITFCQSIISTLTGGGGSGGGGSGGGGSGGGGSGGGGSELCDDDPPEIPHATFKAMAYKEGTMLNCECKRGFRRIKSGSLYMLCTGNSSHSSWDNQCQCTSSATRNTTKQVTPQPEEQKERKTTEMQSPMQPVDQASLPGHCREPPPWENEATERIYHFVVGQMVYYQCVQGYRALHRGPAESVCKMTHGKTRWTQPQLICTGEMETSQFPGEEKPQASPEGRPESETSCLVTTTDFQIQTEMAATMETSIFTTEYQ

SEQ ID NO: 39 - protein, 377 aa, Artificial Sequence
  Synthesized mature form of human IL-2 (Gly4Ser)5- extracellular domain of IL-2 R
APTSSSTKKTQLQLEHLLLDLQMILNGINNYKNPKLTRMLTFKFYMPKKATELKHLQCLEEELKPLEEVLNLAQSKNFHLRPRDLISNINVIVLELKGSETTFMCEYADETATIVEFLNRWITFCQSIISTLTGGGGSGGGGSGGGGSGGGGSGGGGSELCDDDPPEIPHATFKAMAYKEGTMLNCECKRGFRRIKSGSLYMLCTGNSSHSSWDNQCQCTSSATRNTTKQVTPQPEEQKERKTTEMQSPMQPVDQASLPGHCREPPPWENEATERIYHFVVGQMVYYQCVQGYRALHRGPAESVCKMTHGKTRWTQPQLICTGEMETSQFPGEEKPQASPEGRPESETSCLVTTTDFQIQTEMAATMETSIFTTEYQ

SEQ ID NO: 40 - protein, 20 aa, Artificial Sequence
  Linker sequence (Gly4Ser)4
GGGGSGGGGSGGGGSGGGGS

SEQ ID NO: 41 - protein, 25 aa, Artificial Sequence
  Linker sequence (Gly4Ser)5
GGGGSGGGGSGGGGSGGGGSGGGGS

SEQ ID NO: 42 - DNA, 1215 bp, Artificial Sequence
  Synthesized unprocessed form IL-2 (Gly3Ser)3- extracellular domain of IL-2 R
atggacagcatgcagctcgcatcctgtgtcacattgacacttgtgctccttgtcaacagcgcacccacttcaagctctacttcaagctctacagcggaagcacagcagcagcagcagcagcagcagcagcagcagcacctggagcagctgttgatggacctacaggagctcctgagcaggatggagaattacaggaacctgaaactccccaggatgctcaccttcaaattttacttgcccaagcaggccacagaattgaaagatcttcagtgcctagaagatgaacttggacctctgcggcatgttctggatttgactcaaagcaaaagctttcaattggaagatgctgagaatttcatcagcaatatcagagtaactgttgtaaaactaaagggctctgacaacacatttgagtgccaattcgatgatgagtcagcaactgtggtggactttctgaggagatggatagccttctgtcaaagcatcatctcaacaagccctcaaggtggaggttctggtggaggttcaggtggaggttcggaactgtgtctgtatgacccacccgaggtccccaatgccacattcaaagccctctcctacaagaacggcaccatcctaaactgtgaatgcaagagaggtttccgaagactaaaggaattggtctatatgcgttgcttaggaaactcctggagcagcaactgccagtgcaccagcaactcccatgacaaatcgagaaagcaagttacagctcaacttgaacaccagaaagagcaacaaaccacaacagacatgcagaagccaacacagtctatgcaccaagagaaccttacaggtcactgcagggagccacctccttggaaacatgaagattccaagagaatctatcatttcgtggaaggacagagtgttcactacgagtgtattccgggatacaaggctctacagagaggtcctgctattagcatctgcaagatgaagtgtgggaaaacggggtggactcagccccagctcacatgtgtagatgaaagagaacaccaccgatttctggctagtgaggaatctcaaggaagcagaaattcttctcccgagagtgagacttcctgccccataaccaccacagacttcccacaacccacagaaacaactgcaatgacggagacatttgtgctcacaatggagtataagggtggacatcaccatcaccatcactaataa

SEQ ID NO: 43 - protein, 360 aa, Artificial Sequence
  Synthesized mature form IL-2 (Gly3Ser)2- extracellular domain of IL-2 R
APTSSSTKKTQLQLEHLLLDLQMILNGINNYKNPKLTRMLTFKFYMPKKATELKHLQCLEEELKPLEEVLNLAQSKNFHLRPRDLISNINVIVLELKGSETTFMCEYADETATIVEFLNRWITFCQSIISTLTGGGSGGGSELCDDDPPEIPHATFKAMAYKEGTMLNCECKRGFRRIKSGSLYMLCTGNSSHSSWDNQCQCTSSATRNTTKQVTPQPEEQKERKTTEMQSPMQPVDQASLPGHCREPPPWENEATERIYHFVVGQMVYYQCVQGYRALHRGPAESVCKMTHGKTRWTQPQLICTGEMETSQFPGEEKPQASPEGRPESETSCLVTTTDFQIQTEMAATMETSIFTTEYQ

SEQ ID NO: 44 - protein, 380 aa, Artificial Sequence
  Synthesized unprocessed form IL-2 (Gly3Ser)2- extracellular domain of IL-2 R
MDRMQLLSCIALSLALVTNSAPTSSSTKKTQLQLEHLLLDLQMILNGINNYKNPKLTRMLTFKFYMPKKATELKHLQCLEEELKPLEEVLNLAQSKNFHLRPRDLISNINVIVLELKGSETTFMCEYADETATIVEFLNRWITFCQSIISTLTGGGSGGGSELCDDDPPEIPHATFKAMAYKEGTMLNCECKRGFRRIKSGSLYMLCTGNSSHSSWDNQCQCTSSATRNTTKQVTPQPEEQKERKTTEMQSPMQPVDQASLPGHCREPPPWENEATERIYHFVVGQMVYYQCVQGYRALHRGPAESVCKMTHGKTRWTQPQLICTGEMETSQFPGEEKPQASPEGRPESETSCLVTTTDFQIQTEMAATMETSIFTTEYQ

SEQ ID NO: 45 - protein, 355 aa, Artificial Sequence
  Synthesized mature form IL-2 (Gly3)- extracellular domain of IL-2 R
APTSSSTKKTQLQLEHLLLDLQMILNGINNYKNPKLTRMLTFKFYMPKKATELKHLQCLEEELKPLEEVLNLAQSKNFHLRPRDLISNINVIVLELKGSETTFMCEYADETATIVEFLNRWITFCQSIISTLTGGGELCDDDPPEIPHATFKAMAYKEGTMLNCECKRGFRRIKSGSLYMLCTGNSSHSSWDNQCQCTSSATRNTTKQVTPQPEEQKERKTTEMQSPMQPVDQASLPGHCREPPPWENEATERIYHFVVGQMVYYQCVQGYRALHRGPAESVCKMTHGKTRWTQPQLICTGEMETSQFPGEEKPQASPEGRPESETSCLVTTTDFQIQTEMAATMETSIFTTEYQ

SEQ ID NO: 46 - protein, 375 aa, Artificial Sequence
  Synthesized unprocessed form IL-2 (Gly3)- extracellular domain of IL-2 R
MDRMQLLSCIALSLALVTNSAPTSSSTKKTQLQLEHLLLDLQMILNGINNYKNPKLTRMLTFKFYMPKKATELKHLQCLEEELKPLEEVLNLAQSKNFHLRPRDLISNINVIVLELKGSETTFMCEYADETATIVEFLNRWITFCQSIISTLTGGGELCDDDPPEIPHATFKAMAYKEGTMLNCECKRGFRRIKSGSLYMLCTGNSSHSSWDNQCQCTSSATRNTTKQVTPQPEEQKERKTTEMQSPMQPVDQASLPGHCREPPPWENEATERIYHFVVGQMVYYQCVQGYRALHRGPAESVCKMTHGKTRWTQPQLICTGEMETSQFPGEEKPQASPEGRPESETSCLVTTTDFQIQTEMAATMETSIFTTEYQ

SEQ ID NO: 47 - DNA, 1170 bp, Artificial Sequence
  Synthesized unprocessed form IL-2 (Gly3Ser)2- extracellular domain of IL-2 R
atggacaggatgcaactcctgtcttgcattgcactaagtcttgcacttgtcacaaacagtgcacctacttcaagttctacaaagaaaacacagctacaactggagcatttactgctggatttacagatgattttgaatggaattaataattacaagaatcccaaactcaccaggatgctcacatttaagttttacatgcccaagaaggccacagaactgaaacatcttcagtgtctagaagaagaactcaaacctctggaggaagtgctaaatttagctcaaagcaaaaactttcacttaagacccagggacttaatcagcaatatcaacgtaatagttctggaactaaagggatctgaaacaacattcatgtgtgaatatgctgatgagacagcaaccattgtagaatttctgaacagatggattaccttttgtcaaagcatcatctcaacactgactggtggaggttctggtggaggttcagagctctgtgacgatgacccgccagagatcccacacgccacattcaaagccatggcctacaaggaaggaaccatgttgaactgtgaatgcaagagaggtttccgcagaataaaaagcgggtcactctatatgctctgtacaggaaactctagccactcgtcctgggacaaccaatgtcaatgcacaagctctgccactcggaacacaacgaaacaagtgacacctcaacctgaagaacagaaagaaaggaaaaccacagaaatgcaaagtccaatgcagccagtggaccaagcgagccttccaggtcactgcagggaacctccaccatgggaaaatgaagccacagagagaatttatcatttcgtggtggggcagatggtttattatcagtgcgtccagggatacagggctctacacagaggtcctgctgagagcgtctgcaaaatgacccacgggaagacaaggtggacccagccccagctcatatgcacaggtgaaatggagaccagtcagtttccaggtgaagagaagcctcaggcaagccccgaaggccgtcctgagagtgagacttcctgcctcgtcacaacaacagattttcaaatacagacagaaatggctgcaaccatggagacgtccatatttacaacagagtaccagggtggacatcaccatcaccatcactaataa

SEQ ID NO: 48 - DNA, 1155 bp, Artificial Sequence
  Synthesized unprocessed form IL-2 (Gly3)- extracellular domain of IL-2 R
atggacaggatgcaactcctgtcttgcattgcactaagtcttgcacttgtcacaaacagtgcacctacttcaagttctacaaagaaaacacagctacaactggagcatttactgctggatttacagatgattttgaatggaattaataattacaagaatcccaaactcaccaggatgctcacatttaagttttacatgcccaagaaggccacagaactgaaacatcttcagtgtctagaagaagaactcaaacctctggaggaagtgctaaatttagctcaaagcaaaaactttcacttaagacccagggacttaatcagcaatatcaacgtaatagttctggaactaaagggatctgaaacaacattcatgtgtgaatatgctgatgagacagcaaccattgtagaatttctgaacagatggattaccttttgtcaaagcatcatctcaacactgactggtggaggtgagctctgtgacgatgacccgccagagatcccacacgccacattcaaagccatggcctacaaggaaggaaccatgttgaactgtgaatgcaagagaggtttccgcagaataaaaagcgggtcactctatatgctctgtacaggaaactctagccactcgtcctgggacaaccaatgtcaatgcacaagctctgccactcggaacacaacgaaacaagtgacacctcaacctgaagaacagaaagaaaggaaaaccacagaaatgcaaagtccaatgcagccagtggaccaagcgagccttccaggtcactgcagggaacctccaccatgggaaaatgaagccacagagagaatttatcatttcgtggtggggcagatggtttattatcagtgcgtccagggatacagggctctacacagaggtcctgctgagagcgtctgcaaaatgacccacgggaagacaaggtggacccagccccagctcatatgcacaggtgaaatggagaccagtcagtttccaggtgaagagaagcctcaggcaagccccgaaggccgtcctgagagtgagacttcctgcctcgtcacaacaacagattttcaaatacagacagaaatggctgcaaccatggagacgtccatatttacaacagagtaccagggtggacatcaccatcaccatcactaataa

SEQ ID NO: 49 - DNA, 1221 bp, Artificial Sequence
  Synthesized unprocessed form IL-2 (Gly4Ser)5- extracellular domain of IL-2 R
atggacaggatgcaactcctgtcttgcattgcactaagtcttgcacttgtcacaaacagtgcacctacttcaagttctacaaagaaaacacagctacaactggagcatttactgctggatttacagatgattttgaatggaattaataattacaagaatcccaaactcaccaggatgctcacatttaagttttacatgcccaagaaggccacagaactgaaacatcttcagtgtctagaagaagaactcaaacctctggaggaagtgctaaatttagctcaaagcaaaaactttcacttaagacccagggacttaatcagcaatatcaacgtaatagttctggaactaaagggatctgaaacaacattcatgtgtgaatatgctgatgagacagcaaccattgtagaatttctgaacagatggattaccttttgtcaaagcatcatctcaacactgactggtggaggtggatcaggtggaggtggatctggtggaggtggatcaggtggaggtggatccggtggaggtggatctgagctctgtgacgatgacccgccagagatcccacacgccacattcaaagccatggcctacaaggaaggaaccatgttgaactgtgaatgcaagagaggtttccgcagaataaaaagcgggtcactctatatgctctgtacaggaaactctagccactcgtcctgggacaaccaatgtcaatgcacaagctctgccactcggaacacaacgaaacaagtgacacctcaacctgaagaacagaaagaaaggaaaaccacagaaatgcaaagtccaatgcagccagtggaccaagcgagccttccaggtcactgcagggaacctccaccatgggaaaatgaagccacagagagaatttatcatttcgtggtggggcagatggtttattatcagtgcgtccagggatacagggctctacacagaggtcctgctgagagcgtctgcaaaatgacccacgggaagacaaggtggacccagccccagctcatatgcacaggtgaaatggagaccagtcagtttccaggtgaagagaagcctcaggcaagccccgaaggccgtcctgagagtgagacttcctgcctcgtcacaacaacagattttcaaatacagacagaaatggctgcaaccatggagacgtccatatttacaacagagtaccagggtggacatcaccatcaccatcactaataa

SEQ ID NO: 50 - protein, 15 aa, Artificial Sequence
  (Gly4Ser)3 linker
GGGGSGGGGSGGGGS

SEQ ID NO: 51 - protein, 10 aa, Artificial Sequence
  (Gly4Ser)2 linker
GGGGSGGGGS

SEQ ID NO: 52 - protein, 5 aa, Artificial Sequence
  (Gly4Ser)1 linker
GGGGS

SEQ ID NO: 53 - DNA, 10 bp, Artificial Sequence
  Kozak sequence
gccaccatgg

SEQ ID NO: 54 - protein, 412 aa, Artificial Sequence
  Synthesized unprocessed form of IL-2 (Gly4Ser)4-extracellular domain of IL-2 R + glycine spacer and poly-histidine region
MDSMQLASCVTLTLVLLVNSAPTSSSTSSSTAEAQQQQQQQQQQQQHLEQLLMDLQELLSRMENYRNLKLPRMLTFKFYLPKQATELKDLQCLEDELGPLRHVLDLTQSKSFQLEDAENFISNIRVTVVKLKGSDNTFECQFDDESATVVDFLRRWIAFCQSIISTSPQGGGGSGGGGSGGGGSGGGGSELCLYDPPEVPNATFKALSYKNGTILNCECKRGFRRLKELVYMRCLGNSWSSNCQCTSNSHDKSRKQVTAQLEHQKEQQTTTDMQKPTQSMHQENLTGHCREPPPWKHEDSKRIYHFVEGQSVHYECIPGYKALQRGPAISICKMKCGKTGWTQPQLTCVDEREHHRFLASEESQGSRNSSPESETSCPITTTDFPQPTETTAMTETFVLTMEYKGGHHHHHH

SEQ ID NO: 55 - protein, 417 aa, Artificial Sequence
  Synthesized unprocessed form of IL-2 (Gly4Ser)5- extracellular domain of IL-2 R + glycine spacer and poly-histidine region
MDSMQLASCVTLTLVLLVNSAPTSSSTSSSTAEAQQQQQQQQQQQQHLEQLLMDLQELLSRMENYRNLKLPRMLTFKFYLPKQATELKDLQCLEDELGPLRHVLDLTQSKSFQLEDAENFISNIRVTVVKLKGSDNTFECQFDDESATVVDFLRRWIAFCQSIISTSPQGGGGSGGGGSGGGGSGGGGSGGGGSELCLYDPPEVPNATFKALSYKNGTILNCECKRGFRRLKELVYMRCLGNSWSSNCQCTSNSHDKSRKQVTAQLEHQKEQQTTTDMQKPTQSMHQENLTGHCREPPPWKHEDSKRIYHFVEGQSVHYECIPGYKALQRGPAISICKMKCGKTGWTQPQLTCVDEREHHRFLASEESQGSRNSSPESETSCPITTTDFPQPTETTAMTETFVLTMEYKGGHHHHHH

SEQ ID NO: 56 - protein, 408 aa, Artificial Sequence
  Synthesized unprocessed form of IL-2 (Gly3Ser)4- extracellular domain of IL-2 R + glycine spacer and poly-histidine region
MDSMQLASCVTLTLVLLVNSAPTSSSTSSSTAEAQQQQQQQQQQQQHLEQLLMDLQELLSRMENYRNLKLPRMLTFKFYLPKQATELKDLQCLEDELGPLRHVLDLTQSKSFQLEDAENFISNIRVTVVKLKGSDNTFECQFDDESATVVDFLRRWIAFCQSIISTSPQGGGSGGGSGGGSGGGSELCLYDPPEVPNATFKALSYKNGTILNCECKRGFRRLKELVYMRCLGNSWSSNCQCTSNSHDKSRKQVTAQLEHQKEQQTTTDMQKPTQSMHQENLTGHCREPPPWKHEDSKRIYHFVEGQSVHYECIPGYKALQRGPAISICKMKCGKTGWTQPQLTCVDEREHHRFLASEESQGSRNSSPESETSCPITTTDFPQPTETTAMTETFVLTMEYKGGHHHHHH

SEQ ID NO: 57 - protein, 404 aa, Artificial Sequence
  Synthesized unprocessed form of IL-2 (Gly3Ser)3- extracellular domain of IL-2 R + glycine spacer and poly-histidine region
MDSMQLASCVTLTLVLLVNSAPTSSSTSSSTAEAQQQQQQQQQQQQHLEQLLMDLQELLSRMENYRNLKLPRMLTFKFYLPKQATELKDLQCLEDELGPLRHVLDLTQSKSFQLEDAENFISNIRVTVVKLKGSDNTFECQFDDESATVVDFLRRWIAFCQSIISTSPQGGGSGGGSGGGSELCLYDPPEVPNATFKALSYKNGTILNCECKRGFRRLKELVYMRCLGNSWSSNCQCTSNSHDKSRKQVTAQLEHQKEQQTTTDMQKPTQSMHQENLTGHCREPPPWKHEDSKRIYHFVEGQSVHYECIPGYKALQRGPAISICKMKCGKTGWTQPQLTCVDEREHHRFLASEESQGSRNSSPESETSCPITTTDFPQPTETTAMTETFVLTMEYKGGHHHHHH

SEQ ID NO: 58 - protein, 388 aa, Artificial Sequence
  Synthesized unprocessed form IL-2 (Gly3Ser)2- extracellular domain of IL-2 R + glycine spacer and poly-histidine region
MDRMQLLSCIALSLALVTNSAPTSSSTKKTQLQLEHLLLDLQMILNGINNYKNPKLTRMLTFKFYMPKKATELKHLQCLEEELKPLEEVLNLAQSKNFHLRPRDLISNINVIVLELKGSETTFMCEYADETATIVEFLNRWITFCQSIISTLTGGGSGGGSELCDDDPPEIPHATFKAMAYKEGTMLNCECKRGFRRIKSGSLYMLCTGNSSHSSWDNQCQCTSSATRNTTKQVTPQPEEQKERKTTEMQSPMQPVDQASLPGHCREPPPWENEATERIYHFVVGQMVYYQCVQGYRALHRGPAESVCKMTHGKTRWTQPQLICTGEMETSQFPGEEKPQASPEGRPESETSCLVTTTDFQIQTEMAATMETSIFTTEYQGGHHHHHH

SEQ ID NO: 59 - protein, 392 aa, Artificial Sequence
  Synthesized unprocessed form of IL-2 (Gly3Ser)3- extracellular domain of IL-2 R + glycine spacer and poly-histidine region
MDRMQLLSCIALSLALVTNSAPTSSSTKKTQLQLEHLLLDLQMILNGINNYKNPKLTRMLTFKFYMPKKATELKHLQCLEEELKPLEEVLNLAQSKNFHLRPRDLISNINVIVLELKGSETTFMCEYADETATIVEFLNRWITFCQSIISTLTGGGSGGGSGGGSELCDDDPPEIPHATFKAMAYKEGTMLNCECKRGFRRIKSGSLYMLCTGNSSHSSWDNQCQCTSSATRNTTKQVTPQPEEQKERKTTEMQSPMQPVDQASLPGHCREPPPWENEATERIYHFVVGQMVYYQCVQGYRALHRGPAESVCKMTHGKTRWTQPQLICTGEMETSQFPGEEKPQASPEGRPESETSCLVTTTDFQIQTEMAATMETSIFTTEYQGGHHHHHH

SEQ ID NO: 60 - protein, 396 aa, Artificial Sequence
  Synthesized unprocessed form IL-2 (Gly3Ser)4- extracellular domain of IL-2 R + glycine spacer and poly-histidine region
MDRMQLLSCIALSLALVTNSAPTSSSTKKTQLQLEHLLLDLQMILNGINNYKNPKLTRMLTFKFYMPKKATELKHLQCLEEELKPLEEVLNLAQSKNFHLRPRDLISNINVIVLELKGSETTFMCEYADETATIVEFLNRWITFCQSIISTLTGGGSGGGSGGGSGGGSELCDDDPPEIPHATFKAMAYKEGTMLNCECKRGFRRIKSGSLYMLCTGNSSHSSWDNQCQCTSSATRNTTKQVTPQPEEQKERKTTEMQSPMQPVDQASLPGHCREPPPWENEATERIYHFVVGQMVYYQCVQGYRALHRGPAESVCKMTHGKTRWTQPQLICTGEMETSQFPGEEKPQASPEGRPESETSCLVTTTDFQIQTEMAATMETSIFTTEYQGGHHHHHH

SEQ ID NO: 61 - protein, 400 aa, Artificial Sequence
  Synthesized unprocessed form IL-2 (Gly4Ser)4- extracellular domain of IL-2 R + glycine spacer and poly-histidine region
MDRMQLLSCIALSLALVTNSAPTSSSTKKTQLQLEHLLLDLQMILNGINNYKNPKLTRMLTFKFYMPKKATELKHLQCLEEELKPLEEVLNLAQSKNFHLRPRDLISNINVIVLELKGSETTFMCEYADETATIVEFLNRWITFCQSIISTLTGGGGSGGGGSGGGGSGGGGSELCDDDPPEIPHATFKAMAYKEGTMLNCECKRGFRRIKSGSLYMLCTGNSSHSSWDNQCQCTSSATRNTTKQVTPQPEEQKERKTTEMQSPMQPVDQASLPGHCREPPPWENEATERIYHFVVGQMVYYQCVQGYRALHRGPAESVCKMTHGKTRWTQPQLICTGEMETSQFPGEEKPQASPEGRPESETSCLVTTTDFQIQTEMAATMETSIFTTEYQGGHHHHHH

SEQ ID NO: 62 - protein, 364 aa, Artificial Sequence
  Synthesized mature form IL-2 (Gly3Ser)3- extracellular domain of mutIL-2 R
APTSSSTKKTQLQLEHLLLDLQMILNGINNYKNPKLTRMLTFKFYMPKKATELKHLQCLEEELKPLEEVLNLAQSKNFHLRPRDLISNINVIVLELKGSETTFMCEYADETATIVEFLNRWITFCQSIISTLTGGGSGGGSGGGSELCDDDPPEIPHATFKAMAYKEGTMLNCECKRGFTSIKSGSLYMLCTGNSSHSSWDNQCQCTSSATRNTTKQVTPQPEEQKERKTTEMQSPMQPVDQASLPGHCREPPPWENEATERIYHFVVGQMVYYQCVQGYRALHRGPAESVCKMTHGKTRWTQPQLICTGEMETSQFPGEEKPQASPEGRPESETSCLVTTTDFQIQTEMAATMETSIFTTEYQ

SEQ ID NO: 63 - DNA, 1182 bp, Artificial Sequence
  Synthesized unprocessed form IL-2 (Gly3Ser)3- extracellular domain of mutIL-2 R Mut
atggacaggatgcaactcctgtcttgcattgcactaagtcttgcacttgtcacaaacagtgcacctacttcaagttctacaaagaaaacacagctacaactggagcatttactgctggatttacagatgattttgaatggaattaataattacaagaatcccaaactcaccaggatgctcacatttaagttttacatgcccaagaaggccacagaactgaaacatcttcagtgtctagaagaagaactcaaacctctggaggaagtgctaaatttagctcaaagcaaaaactttcacttaagacccagggacttaatcagcaatatcaacgtaatagttctggaactaaagggatctgaaacaacattcatgtgtgaatatgctgatgagacagcaaccattgtagaatttctgaacagatggattaccttttgtcaaagcatcatctcaacactgactggtggaggttctggtggaggttcaggtggaggttcggagctctgtgacgatgacccgccagagatcccacacgccacattcaaagccatggcctacaaggaaggaaccatgttgaactgtgaatgcaagagaggtttcacctcaataaaaagcgggtcactctatatgctctgtacaggaaactctagccactcgtcctgggacaaccaatgtcaatgcacaagctctgccactcggaacacaacgaaacaagtgacacctcaacctgaagaacagaaagaaaggaaaaccacagaaatgcaaagtccaatgcagccagtggaccaagcgagccttccaggtcactgcagggaacctccaccatgggaaaatgaagccacagagagaatttatcatttcgtggtggggcagatggtttattatcagtgcgtccagggatacagggctctacacagaggtcctgctgagagcgtctgcaaaatgacccacgggaagacaaggtggacccagccccagctcatatgcacaggtgaaatggagaccagtcagtttccaggtgaagagaagcctcaggcaagccccgaaggccgtcctgagagtgagacttcctgcctcgtcacaacaacagattttcaaatacagacagaaatggctgcaaccatggagacgtccatatttacaacagagtaccagggtggacatcaccatcaccatcactaataa

SEQ ID NO: 64 - protein, 372 aa, Artificial Sequence
  Synthesized mature form IL-2 (Gly4Ser)4- extracellular domain of mutIL-2 R
APTSSSTKKTQLQLEHLLLDLQMILNGINNYKNPKLTRMLTFKFYMPKKATELKHLQCLEEELKPLEEVLNLAQSKNFHLRPRDLISNINVIVLELKGSETTFMCEYADETATIVEFLNRWITFCQSIISTLTGGGGSGGGGSGGGGSGGGGSELCDDDPPEIPHATFKAMAYKEGTMLNCECKRGFTSIKSGSLYMLCTGNSSHSSWDNQCQCTSSATRNTTKQVTPQPEEQKERKTTEMQSPMQPVDQASLPGHCREPPPWENEATERIYHFVVGQMVYYQCVQGYRALHRGPAESVCKMTHGKTRWTQPQLICTGEMETSQFPGEEKPQASPEGRPESETSCLVTTTDFQIQTEMAATMETSIFTTEYQ

SEQ ID NO: 65 - DNA, 1206 bp, Artificial Sequence
  Synthesized unprocessed form IL-2 (Gly4Ser)4- extracellular domain of mutIL-2 R
atggacaggatgcaactcctgtcttgcattgcactaagtcttgcacttgtcacaaacagtgcacctacttcaagttctacaaagaaaacacagctacaactggagcatttactgctggatttacagatgattttgaatggaattaataattacaagaatcccaaactcaccaggatgctcacatttaagttttacatgcccaagaaggccacagaactgaaacatcttcagtgtctagaagaagaactcaaacctctggaggaagtgctaaatttagctcaaagcaaaaactttcacttaagacccagggacttaatcagcaatatcaacgtaatagttctggaactaaagggatctgaaacaacattcatgtgtgaatatgctgatgagacagcaaccattgtagaatttctgaacagatggattaccttttgtcaaagcatcatctcaacactgactggtggaggtggatctggtggaggtggatcaggtggaggtggatccggtggaggtggatctgagctctgtgacgatgacccgccagagatcccacacgccacattcaaagccatggcctacaaggaaggaaccatgttgaactgtgaatgcaagagaggtttcacctcaataaaaagcgggtcactctatatgctctgtacaggaaactctagccactcgtcctgggacaaccaatgtcaatgcacaagctctgccactcggaacacaacgaaacaagtgacacctcaacctgaagaacagaaagaaaggaaaaccacagaaatgcaaagtccaatgcagccagtggaccaagcgagccttccaggtcactgcagggaacctccaccatgggaaaatgaagccacagagagaatttatcatttcgtggtggggcagatggtttattatcagtgcgtccagggatacagggctctacacagaggtcctgctgagagcgtctgcaaaatgacccacgggaagacaaggtggacccagccccagctcatatgcacaggtgaaatggagaccagtcagtttccaggtgaagagaagcctcaggcaagccccgaaggccgtcctgagagtgagacttcctgcctcgtcacaacaacagattttcaaatacagacagaaatggctgcaaccatggagacgtccatatttacaacagagtaccagggtggacatcaccatcaccatcactaataa